European Patent Application EP 4 722 367 A1, published April 8, 2026. Title: mRNA structure platform for protein expression with high efficiency. Applicant: KOREA RESEARCH INSTITUTE OF BIOSCIENCE AND BIOTECHNOLOGY. The sequence listing filed with the application follows.

SEQUENCE LISTING (29 sequences)

SEQ ID NO: 1 - DNA, 639 bp, synthetic construct
  source 1..639: mol_type = other DNA
atggtcttcacactcgaagatttcgttggggactggcgacagacagccggctacaacctggaccaagtccttgaacagggaggtgtgtccagtttgtttcagaatctcggggtgtccgtaactccgatccaaaggattgtcctgagcggtgaaaatgggctgaagatcgacatccatgtcatcatcccgtatgaaggtctgagcggcgaccaaatgggccagatcgaaaaaatttttaaggtggtgtaccctgtggatgatcatcactttaaggtgatcctgcactatggcacactggtaatcgacggggttacgccgaacatgatcgactatttcggacggccgtatgaaggcatcgccgtgttcgacggcaaaaagatcactgtaacagggaccctgtggaacggcaacaaaattatcgacgagcgcctgatcaaccccgacggctccctgctgttccgagtaaccatcaacggagtgaccggctggcggctgtgcgaacgcattctggcgaattctcacggcttccctcccgaggtggaggagcaggccgccggcaccctgcccatgagctgcgcccaggagagcggcatggatagacaccctgctgcttgcgccagcgccaggatcaacgtctaa

SEQ ID NO: 2 - DNA, 43 bp, synthetic construct
  source 1..43: mol_type = other DNA
actcttctggtccccacagactcagagagaaccccttaagacc

SEQ ID NO: 3 - DNA, 111 bp, synthetic construct
  source 1..111: mol_type = other DNA
gctggagcctcggtggccatgcttcttgccccttgggcctccccccagcccctcctccccttcctgcacccgtacccccgtggtctttgaataaagtctgagtgggcggca

SEQ ID NO: 4 - DNA, 134 bp, synthetic construct
  source 1..134: mol_type = other DNA
gctcgctttcttgctgtccaatttctattaaaggttcctttgttccctaagtccaactactaaactgggggatattatgaagggccttgagcatctggattctgcctaataaaaaacatttattttcattgcaa

SEQ ID NO: 5 - DNA, 90 bp, synthetic construct
  source 1..90: mol_type = other DNA
gctcactgcccatgattcagagctttcaaggataggctttattctgcaagcaatacaaataataaatctattctgctgagagatcacaca

SEQ ID NO: 6 - DNA, 103 bp, synthetic construct
  source 1..103: mol_type = other DNA
gcgccgcctccgggacccccaggacaggctgcggcccctcccccgtcctggaggttccccagccccacttaccgcgtaatgcgccaataaaccaatgaacgaa

SEQ ID NO: 7 - DNA, 304 bp, synthetic construct
  source 1..304: mol_type = other DNA
gtgcacggcgtccctgagggcccttcccaacctcccctggtcctgcactgtcccggagctcaggccctggtgaggggctgggtcccgggtgccccccatgccctccctgctgccaggctcccactgcccctgcacctgcttctcagcgcaacagctgtgtgtgcccgtggtgaggttgtgctgcctgtggtgaggtcctgtcctggctcccagggtcctgggggctgctgcactgccctccgcccttccctgacactgtctgctgccccaatcaccgtcacaataaaagaaactgtggtctcta

SEQ ID NO: 8 - DNA, 73 bp, synthetic construct
  source 1..73: mol_type = other DNA
acgcagcccgcaggcagccccacacccgccgcctcctgcaccgagagagatggaataaagcccttgaaccagc

SEQ ID NO: 9 - DNA, 190 bp, synthetic construct
  source 1..190: mol_type = other DNA
tgttttggctgggttcttccttgttcgcaccggacacctccagtgaccagacggcaaggttcttatcccagtgtatattggaaaaacatgttatacttttgacaatttaacgtgcctagagctcaaattaaactaataccataacgtaatgcaacttacaacataaataaaggtcaatgtttaatccata

SEQ ID NO: 10 - DNA, 269 bp, synthetic construct
  source 1..269: mol_type = other DNA
tgttttggctgggttcttccttgttcgcaccggacacctccagtgaccagacggcaaggttcttatcccagtgtatatttgttttggctgggttcttccttgttcgcaccggacacctccagtgaccagacggcaaggttcttatcccagtgtatattggaaaaacatgttatacttttgacaatttaacgtgcctagagctcaaattaaactaataccataacgtaatgcaacttacaacataaataaaggtcaatgtttaatccata

SEQ ID NO: 11 - DNA, 348 bp, synthetic construct
  source 1..348: mol_type = other DNA
tgttttggctgggttcttccttgttcgcaccggacacctccagtgaccagacggcaaggttcttatcccagtgtatatttgttttggctgggttcttccttgttcgcaccggacacctccagtgaccagacggcaaggttcttatcccagtgtatatttgttttggctgggttcttccttgttcgcaccggacacctccagtgaccagacggcaaggttcttatcccagtgtatattggaaaaacatgttatacttttgacaatttaacgtgcctagagctcaaattaaactaataccataacgtaatgcaacttacaacataaataaaggtcaatgtttaatccata

SEQ ID NO: 12 - DNA, 742 bp, synthetic construct
  source 1..742: mol_type = other DNA
ttaaaacagcctgtgggttgatcccacccacagggcccattgggcgctagcactctggtatcacggtacctttgtgcgcctgttttataccccctcccccaactgtaacttagaagtaacacacaccgatcaacagtcagcgtggcacaccagccacgttttgatcaagcacttctgttaccccggactgagtatcaatagactgctcacgcggttgaaggagaaagcgttcgttatccggccaactacttcgaaaaacctagtaacaccgtggaagttgcagagtgtttcgctcagcactaccccagtgtagatcaggtcgatgagtcaccgcattccccacgggcgaccgtggcggtggctgcgttggcggcctgcccatggggaaacccatgggacgctctaatacagacatggtgcgaagagtctattgagctagttggtagtcctccggcccctgaatgcggctaatcctaactgcggagcacacaccctcaagccagagggcagtgtgtcgtaacgggcaactctgcagcggaaccgactactttgggtgtccgtgtttcattttattcctatactggctgcttatggtgacaattgagagattgttaccatatagctattggattggccatccggtgactaatagagctattatatatccctttgttgggtttataccacttagcttgaaagaggttaaaacattacaattcattgttaagttgaatacagcaaa

SEQ ID NO: 13 - DNA, 586 bp, synthetic construct
  source 1..586: mol_type = other DNA
cccctctccctcccccccccctaacgttactggccgaagccgcttggaataaggccggtgtgcgtttgtctatatgttattttccaccatattgccgtcttttggcaatgtgagggcccggaaacctggccctgtcttcttgacgagcattcctaggggtctttcccctctcgccaaaggaatgcaaggtctgttgaatgtcgtgaaggaagcagttcctctggaagcttcttgaagacaaacaacgtctgtagcgaccctttgcaggcagcggaaccccccacctggcgacaggtgcctctgcggccaaaagccacgtgtataagatacacctgcaaaggcggcacaaccccagtgccacgttgtgagttggatagttgtggaaagagtcaaatggctctcctcaagcgtattcaacaaggggctgaaggatgcccagaaggtaccccattgtatgggatctgatctggggcctcggtgcacatgctttacatgtgtttagtcgaggttaaaaaacgtctaggccccccgaaccacggggacgtggttttcctttgaaaaacacgatgataatatggccacaacc

SEQ ID NO: 14 - DNA, 357 bp, synthetic construct
  source 1..357: mol_type = other DNA
ggcgacactccaccatagatcactcccctgtgaggaactactgtcttcacgcagaaagcgtctagccatggcgttagtatgagtgtcgtgcagcctccaggaccccccctcccgggagagccatagtggtctgcggaaccggtgagtacaccggaattgccaggacgaccgggtcctttcttggattaacccgctcaatgcctggagatttgggcgtgcccccgcgagactgctagccgagtagtgttgggtcgcgaaaggccttgtggtactgcctgatagggtgcttgcgagtgccccgggaggtctcgtagaccgtgcatcatgagcacaaatcctaaacctcaaagaaaaacc

SEQ ID NO: 15 - DNA, 189 bp, synthetic construct
  source 1..189: mol_type = other DNA
aaagcaaaaatgtgatcttgcttgtaaatacaattttgagaggttaataaattacaagtagtgctatttttgtatttaggttagctatttagctttacgttccaggatgcctagtggcagccccacaatatccaggaagccctctctgcggtttttcagattaggtagtcgaaaaacctaagaaattta

SEQ ID NO: 16 - DNA, 121 bp, unidentified
  source 1..121: mol_type = other DNA
aaaaaaaagaaaaaaaaaagaaaaaaaaaagaaaaaaaaaagaaaaaaaaaagaaaaaaaaaagaaaaaaaaaagaaaaaaaaaagaaaaaaaaaagaaaaaaaaaagaaaaaaaaaagaa

SEQ ID NO: 17 - DNA, 121 bp, synthetic construct
  source 1..121: mol_type = other DNA
aaaaaaaaaaaaagaaaaaaaaaaaaaaaaaaaagaaaaaaaaaaaaaaaaaaaagaaaaaaaaaaaaaaaaaaaagaaaaaaaaaaaaaaaaaaaagaaaaaaaaaaaaaaaaaaaagaa

SEQ ID NO: 18 - DNA, 121 bp, synthetic construct
  source 1..121: mol_type = other DNA
aaaaaaaaaaaaaaaaaaaaaaaaagaaaaaaaaaaaaaaaaaaaaaaaaaaaaaagaaaaaaaaaaaaaaaaaaaaaaaaaaaaaagaaaaaaaaaaaaaaaaaaaaaaaaaaaaaagaa

SEQ ID NO: 19 - DNA, 121 bp, synthetic construct
  source 1..121: mol_type = other DNA
aaaaaaaaaaaaaaaaaaaaaaaaaaaaaaaaaaaagaaaaaaaaaaaaaaaaaaaaaaaaaaaaaaaaaaaaaaaagaaaaaaaaaaaaaaaaaaaaaaaaaaaaaaaaaaaaaaaagaa

SEQ ID NO: 20 - DNA, 121 bp, synthetic construct
  source 1..121: mol_type = other DNA
aaaaaaaaaaaaaaaagaaaaaaaaaaaaaaaaaaaaaaaaaaaaaaaaaaaaaaaaaaaaaaaaaagaaaaaaaaaaaaaaaaaaaaaaaaaaaaaaaaaaaaaaaaaaaaaaaaaagaa

SEQ ID NO: 21 - DNA, 121 bp, synthetic construct
  source 1..121: mol_type = other DNA
aaaaaaaaaaaaaaaaaaaaaaaaaaaaaaaaaaaaaaaaaaaaaaaaaaaaaaaaagaaaaaaaaaaaaaaaaaaaaaaaaaaaaaaaaaaaaaaaaaaaaaaaaaaaaaaaaaaaagaa

SEQ ID NO: 22 - DNA, 131 bp, synthetic construct
  source 1..131: mol_type = other DNA
cagcggaaacgagcgaaaaaaaaacagcggaaacgagcgaaaaaaaaacagcggaaacgagcgaaaaaaaaacagcggaaacgagcgaaaaaaaaacagcggaaacgagcgagagagaaccccttaagacc

SEQ ID NO: 23 - DNA, 101 bp, synthetic construct
  source 1..101: mol_type = other DNA
tccggtcgtaaaaaaaaatccggtcgtaaaaaaaaatccggtcgtaaaaaaaaatccggtcgtaaaaaaaaatccggtcgtagagagaaccccttaagacc

SEQ ID NO: 24 - DNA, 39 bp, synthetic construct
  source 1..39: mol_type = other DNA
gttttcgaaacaaataaaacagaaaagcgaacctaaaca

SEQ ID NO: 25 - DNA, 85 bp, synthetic construct
  source 1..85: mol_type = other DNA
aggggccaagtccatacgacaggccccagcccgccagacggagggccgcagaaaggaaggagacacgaccgccccagaaggagga

SEQ ID NO: 26 - DNA, 57 bp, synthetic construct
  source 1..57: mol_type = other DNA
gcccgccagacggagggccgcagaaaggaaggagacacgaccgccccagaaggagga

SEQ ID NO: 27 - DNA, 61 bp, synthetic construct
  source 1..61: mol_type = other DNA
aaaaaaaaaaaaaaaaaaaaaaaaaaaaaaaaaaaaaaaaaaaaaaaaaaaaaaaaaaaag

SEQ ID NO: 28 - DNA, 122 bp, synthetic construct
  source 1..122: mol_type = other DNA
aaaaaaaaaaaaaaaaaaaaaaaaaaaaaaaaaaaaaaaaaaaaaaaaaaaaaaaaaaaagaaaaaaaaaaaaaaaaaaaaaaaaaaaaaaaaaaaaaaaaaaaaaaaaaaaaaaaaaaaag

SEQ ID NO: 29 - DNA, 183 bp, synthetic construct
  source 1..183: mol_type = other DNA
aaaaaaaaaaaaaaaaaaaaaaaaaaaaaaaaaaaaaaaaaaaaaaaaaaaaaaaaaaaagaaaaaaaaaaaaaaaaaaaaaaaaaaaaaaaaaaaaaaaaaaaaaaaaaaaaaaaaaaaagaaaaaaaaaaaaaaaaaaaaaaaaaaaaaaaaaaaaaaaaaaaaaaaaaaaaaaaaaaaag